European Patent Specification EP 2 817 331 B1, published August 30, 2023. Title: USE OF THE CD2 SIGNALING DOMAIN IN SECOND-GENERATION CHIMERIC ANTIGEN RECEPTORS. Applicant: The Trustees of University of Pennsylvania June, Carl H Scholler, John Posey, Avery D Jr. The sequence listing filed with the application follows.

SEQUENCE LISTING (1 sequence)

SEQ ID NO: 1 - DNA, 1691 bp, Artificial Sequence
  Chemically Synthesized
atggccttaccagtgaccgccttgctcctgccgctggccttgctgctccacgccgccaggccggacatccagatgacacagactacatcctccctgtctgcctctctgggagacagagtcaccatcagttgcagggcaagtcaggacattagtaaatatttaaattggtatcagcagaaaccagatggaactgttaaactcctgatctaccatacatcaagattacactcaggagtcccatcaaggttcagtggcagtgggtctggaacagattattctctcaccattagcaacctggagcaagaagatattgccacttacttttgccaacagggtaatacgcttccgtacacgttcggaggggggaccaagctggagatcacaggtggcggtggctcgggcggtggtgggtcgggtggcggcggatctgaggtgaaactgcaggagtcaggacctggcctggtggcgccctcacagagcctgtccgtcacatgcactgtctcaggggtctcattacccgactatggtgtaagctggattcgccagcctccacgaaagggtctggagtggctgggagtaatatggggtagtgaaaccacatactataattcagctctcaaatccagactgaccatcatcaaggacaactccaagagccaagttttcttaaaaatgaacagtctgcaaactgatgacacagccatttactactgtgccaaacattattactacggtggtagctatgctatggactactggggccaaggaacctcagtcaccgtctcctcaccacgacgccagcgccgcgaccaccaacaccggcgcccaccatcgcgtcgcggcccctgtccctgcgcccagaggcgtgccggccagcggcggggggcgcagtgcacacgagggggctggacttcgcctgtgatatctacatctgggcgcccttggccgggacttgtggggtccttctcctgtcactggttatcaccctttactgcaccaaaaggaaaaaacagaggagtcggagaaatgatgaggagctggagacaagagcccacagagtagctactgaagaaaggggccggaagccccaccaaattccagcttcaacccctcagaatccagcaacttcccaacatcctcctccaccacctggtcatcgttcccaggcacctagtcatcgtcccccgcctcctggacaccgtgttcagcaccagcctcagaagaggcctcctgctccgtcgggcacacaagttcaccagcagaaaggcccgcccctccccagacctcgagttcagccaaaacctccccatggggcagcagaaaactcattgtccccttcctctaatatcgatagagtgaagttcagcaggagcgcagacgcccccgcgtaccagcagggccagaaccagctctataacgagctcaatctaggacgaagagaggagtacgatgttttggacaagagacgtggccgggaccctgagatggggggaaagccgagaaggaagaaccctcaggaaggcctgtacaatgaactgcagaaagataagatggcggaggcctacagtgagattgggatgaaaggcgagcgccggaggggcaaggggcacgatggcctttaccagggtctcagtacagccaccaaggacacctacgacgcccttcacatgcaggccctgccccctcgctaa